European Patent Specification EP 3 286 323 B1, published January 18, 2023. Title: MULTIPLEX DETECTION OF VULVOVAGINAL CANDIDIASIS, TRICHOMONIASIS AND BACTERIAL VAGINOSIS. Applicant: Paquette, Nancy Tremblay, Marie-Helene Tremblay, Simon Therrien, Roseline Belley-Montfort, Lucile Fortin, Marie-Christine Cantin, Dany Roger-Dalbert, Celine. The sequence listing filed with the application follows.

SEQUENCE LISTING (182 sequences)

SEQ ID NO: 1 - DNA, 20 bp, Artificial Sequence
  Synthetic oligonucleotide
ccctatccgctcctgatacc

SEQ ID NO: 2 - DNA, 20 bp, Artificial Sequence
  Synthetic oligonucleotide
ccaaatatctgcgcatttca

SEQ ID NO: 3 - DNA, 23 bp, Artificial Sequence
  Synthetic oligonucleotide
tcccctaccagactcaagcctgc

SEQ ID NO: 4 - DNA, 23 bp, Artificial Sequence
  Synthetic oligonucleotide
gcggctagataagtgtgatgttt

SEQ ID NO: 5 - DNA, 21 bp, Artificial Sequence
  Synthetic oligonucleotide
ctctccagcactcaagctaaa

SEQ ID NO: 6 - DNA, 28 bp, Artificial Sequence
  Synthetic oligonucleotide
caaggcttaaccttggggttcattacaa

SEQ ID NO: 7 - DNA, 21 bp, Artificial Sequence
  Synthetic oligonucleotide
gatgccaacagtatccgtccg

SEQ ID NO: 8 - DNA, 22 bp, Artificial Sequence
  Synthetic oligonucleotide
cctctccgacactcaagttcga

SEQ ID NO: 9 - DNA, 21 bp, Artificial Sequence
  Synthetic oligonucleotide
taccgtaagagaaagccacgg

SEQ ID NO: 10 - DNA, 19 bp, Artificial Sequence
  Synthetic oligonucleotide
gccaacgatgatcgcgtat

SEQ ID NO: 11 - DNA, 19 bp, Artificial Sequence
  Synthetic oligonucleotide
gccaataatgaccgcgtat

SEQ ID NO: 12 - DNA, 19 bp, Artificial Sequence
  Synthetic oligonucleotide
agccgttcactgcggaagt

SEQ ID NO: 13 - DNA, 17 bp, Artificial Sequence
  Synthetic oligonucleotide
acagcactttcgccgcc

SEQ ID NO: 14 - DNA, 18 bp, Artificial Sequence
  Synthetic oligonucleotide
ttaaaaggcggcgtaagc

SEQ ID NO: 15 - DNA, 19 bp, Artificial Sequence
  Synthetic oligonucleotide
gccagttactacctctatc

SEQ ID NO: 16 - DNA, 20 bp, Artificial Sequence
  Synthetic oligonucleotide
aagtctgatggagcaacgcc

SEQ ID NO: 17 - DNA, 23 bp, Artificial Sequence
  Synthetic oligonucleotide
gaagattctggcaagatcaagga

SEQ ID NO: 18 - DNA, 19 bp, Artificial Sequence
  Synthetic oligonucleotide
acgacaatgcagcggatgt

SEQ ID NO: 19 - DNA, 23 bp, Artificial Sequence
  Synthetic oligonucleotide
atcctccgcaactacccacgcca

SEQ ID NO: 20 - DNA, 22 bp, Artificial Sequence
  Synthetic oligonucleotide
cgaacaattgactgaaggtttg

SEQ ID NO: 21 - DNA, 22 bp, Artificial Sequence
  Synthetic oligonucleotide
cggacttcaagaactttggaga

SEQ ID NO: 22 - DNA, 25 bp, Artificial Sequence
  Synthetic oligonucleotide
cttgtaagttcgaagaattgttgga

SEQ ID NO: 23 - DNA, 18 bp, Artificial Sequence
  Synthetic oligonucleotide
ccaccaaagggttgtgac

SEQ ID NO: 24 - DNA, 19 bp, Artificial Sequence
  Synthetic oligonucleotide
cagcatcaccggatttgac

SEQ ID NO: 25 - DNA, 23 bp, Artificial Sequence
  Synthetic oligonucleotide
cggacttgatgaattttggttca

SEQ ID NO: 26 - DNA, 26 bp, Artificial Sequence
  Synthetic oligonucleotide
tgcttgtaaattcgacactttggttg

SEQ ID NO: 27 - DNA, 21 bp, Artificial Sequence
  Synthetic oligonucleotide
gcagcttccttcaatgctcaa

SEQ ID NO: 28 - DNA, 17 bp, Artificial Sequence
  Synthetic oligonucleotide
atcaccagacttgacag

SEQ ID NO: 29 - DNA, 25 bp, Artificial Sequence
  Synthetic oligonucleotide
catgtaagttcgacgaattaatcga

SEQ ID NO: 30 - DNA, 24 bp, Artificial Sequence
  Synthetic oligonucleotide
ggcatggaggttgtcccatttgtg

SEQ ID NO: 31 - DNA, 21 bp, Artificial Sequence
  Synthetic oligonucleotide
ggatctagccgtgtgcccgct

SEQ ID NO: 32 - DNA, 32 bp, Artificial Sequence
  Synthetic oligonucleotide
ttgatgcctcttcacattgctccacctttcct

SEQ ID NO: 33 - DNA, 22 bp, Artificial Sequence
  Synthetic oligonucleotide
gttaggtcaggagttaaatctg

SEQ ID NO: 34 - DNA, 17 bp, Artificial Sequence
  Synthetic oligonucleotide
tcatggcccagaagacc

SEQ ID NO: 35 - DNA, 17 bp, Artificial Sequence
  Synthetic oligonucleotide
tcgtggcccagaaggcc

SEQ ID NO: 36 - DNA, 17 bp, Artificial Sequence
  Synthetic oligonucleotide
ccctggtagtcctagct

SEQ ID NO: 37 - DNA, 17 bp, Artificial Sequence
  Synthetic oligonucleotide
ccctggtagtcctagcc

SEQ ID NO: 38 - DNA, 20 bp, Artificial Sequence
  Synthetic oligonucleotide
cggcacggaaagtataatct

SEQ ID NO: 39 - DNA, 20 bp, Artificial Sequence
  Synthetic oligonucleotide
ggtgaagcagtggaaacact

SEQ ID NO: 40 - DNA, 18 bp, Artificial Sequence
  Synthetic oligonucleotide
ttcgcttctgctcgcgca

SEQ ID NO: 41 - DNA, 18 bp, Artificial Sequence
  Synthetic oligonucleotide
gcagcccaggacataagg

SEQ ID NO: 42 - DNA, 19 bp, Artificial Sequence
  Synthetic oligonucleotide
attcgcttctgctcgcgca

SEQ ID NO: 43 - DNA, 18 bp, Artificial Sequence
  Synthetic oligonucleotide
gcagggacgaggccgcaa

SEQ ID NO: 44 - DNA, 17 bp, Artificial Sequence
  Synthetic oligonucleotide
tcatggcccagaagacc

SEQ ID NO: 45 - DNA, 19 bp, Artificial Sequence
  Synthetic oligonucleotide
cggattcattgggcgtaaa

SEQ ID NO: 46 - DNA, 15 bp, Artificial Sequence
  Synthetic oligonucleotide
cgcctcagcgtcagt

SEQ ID NO: 47 - DNA, 19 bp, Artificial Sequence
  Synthetic oligonucleotide
cggattcattgggcgtaaa

SEQ ID NO: 48 - DNA, 21 bp, Artificial Sequence
  Synthetic oligonucleotide
acacctagtgtccatcgttta

SEQ ID NO: 49 - DNA, 18 bp, Artificial Sequence
  Synthetic oligonucleotide
ccttcgggttgtaaaccg

SEQ ID NO: 50 - DNA, 15 bp, Artificial Sequence
  Synthetic oligonucleotide
cgcctcagcgtcagt

SEQ ID NO: 51 - DNA, 20 bp, Artificial Sequence
  Synthetic oligonucleotide
aggcggctagataagtgtga

SEQ ID NO: 52 - DNA, 22 bp, Artificial Sequence
  Synthetic oligonucleotide
tcctctccagcactcaagctaa

SEQ ID NO: 53 - DNA, 22 bp, Artificial Sequence
  Synthetic oligonucleotide
ttaaccttggggttcattacaa

SEQ ID NO: 54 - DNA, 24 bp, Artificial Sequence
  Synthetic oligonucleotide
aattcagtctcctgaatcgtcaga

SEQ ID NO: 55 - DNA, 20 bp, Artificial Sequence
  Synthetic oligonucleotide
aggcggctagataagtgtga

SEQ ID NO: 56 - DNA, 22 bp, Artificial Sequence
  Synthetic oligonucleotide
cgtgtaggcggctagataagtg

SEQ ID NO: 57 - DNA, 24 bp, Artificial Sequence
  Synthetic oligonucleotide
gaatacttattgtgttaactgcgc

SEQ ID NO: 58 - DNA, 24 bp, Artificial Sequence
  Synthetic oligonucleotide
aagttcgacagtttccgtcccctc

SEQ ID NO: 59 - DNA, 18 bp, Artificial Sequence
  Synthetic oligonucleotide
ggcggcgaaagtgctgta

SEQ ID NO: 60 - DNA, 21 bp, Artificial Sequence
  Synthetic oligonucleotide
caagctcggcatgttatccat

SEQ ID NO: 61 - DNA, 21 bp, Artificial Sequence
  Synthetic oligonucleotide
ggaaacgggtggtaatgctgg

SEQ ID NO: 62 - DNA, 20 bp, Artificial Sequence
  Synthetic oligonucleotide
cgaagcctaggtgggccatt

SEQ ID NO: 63 - DNA, 22 bp, Artificial Sequence
  Synthetic oligonucleotide
ttactggtgtatcactgtaagg

SEQ ID NO: 64 - DNA, 19 bp, Artificial Sequence
  Synthetic oligonucleotide
ccgtcacaggctgaacagt

SEQ ID NO: 65 - DNA, 24 bp, Artificial Sequence
  Synthetic oligonucleotide
ccagaatttgatggataacatgcc

SEQ ID NO: 66 - DNA, 20 bp, Artificial Sequence
  Synthetic oligonucleotide
atggacaatatgccaagcct

SEQ ID NO: 67 - DNA, 20 bp, Artificial Sequence
  Synthetic oligonucleotide
ttcactgcggaagttacaga

SEQ ID NO: 68 - DNA, 20 bp, Artificial Sequence
  Synthetic oligonucleotide
ttaactgcggaagtaacgga

SEQ ID NO: 69 - DNA, 20 bp, Artificial Sequence
  Synthetic oligonucleotide
ttaactgctgaagtaacgga

SEQ ID NO: 70 - DNA, 17 bp, Artificial Sequence
  Synthetic oligonucleotide
acagcactctcgccgcc

SEQ ID NO: 71 - DNA, 24 bp, Artificial Sequence
  Synthetic oligonucleotide
gatagaggtagtaactggccttta

SEQ ID NO: 72 - DNA, 25 bp, Artificial Sequence
  Synthetic oligonucleotide
ctttgtatctctacaaatggcacta

SEQ ID NO: 73 - DNA, 22 bp, Artificial Sequence
  Synthetic oligonucleotide
cgagcttgcctagatgaatttg

SEQ ID NO: 74 - DNA, 20 bp, Artificial Sequence
  Synthetic oligonucleotide
ctctagacatgcgtctagtg

SEQ ID NO: 75 - DNA, 26 bp, Artificial Sequence
  Synthetic oligonucleotide
gatttacttcggtaatgacgttagga

SEQ ID NO: 76 - DNA, 23 bp, Artificial Sequence
  Synthetic oligonucleotide
agctgatcatgcgatctgctttc

SEQ ID NO: 77 - DNA, 27 bp, Artificial Sequence
  Synthetic oligonucleotide
gcctatagaaattcttcggaatggaca

SEQ ID NO: 78 - DNA, 24 bp, Artificial Sequence
  Synthetic oligonucleotide
caaatggtatcccagacttaaggg

SEQ ID NO: 79 - DNA, 18 bp, Artificial Sequence
  Synthetic oligonucleotide
gtcgagcgagcttgccta

SEQ ID NO: 80 - DNA, 26 bp, Artificial Sequence
  Synthetic oligonucleotide
gaactaacagatttacttcggtaatg

SEQ ID NO: 81 - DNA, 22 bp, Artificial Sequence
  Synthetic oligonucleotide
aaactctagacatgcgtctagt

SEQ ID NO: 82 - DNA, 21 bp, Artificial Sequence
  Synthetic oligonucleotide
gtttccaaatggtatcccaga

SEQ ID NO: 83 - DNA, 21 bp, Artificial Sequence
  Synthetic oligonucleotide
gcctagatgaatttggtgctt

SEQ ID NO: 84 - DNA, 23 bp, Artificial Sequence
  Synthetic oligonucleotide
cgagcttgcctatagaaattctt

SEQ ID NO: 85 - DNA, 26 bp, Artificial Sequence
  Synthetic oligonucleotide
gaactaacagatttacttcggtaatg

SEQ ID NO: 86 - DNA, 22 bp, Artificial Sequence
  Synthetic oligonucleotide
aaactctagacatgcgtctagt

SEQ ID NO: 87 - DNA, 21 bp, Artificial Sequence
  Synthetic oligonucleotide
gtttccaaatggtatcccaga

SEQ ID NO: 88 - DNA, 22 bp, Artificial Sequence
  Synthetic oligonucleotide
actagacgcatgtctagagttt

SEQ ID NO: 89 - DNA, 25 bp, Artificial Sequence
  Synthetic oligonucleotide
tgcattagctagttggtaaggtaac

SEQ ID NO: 90 - DNA, 20 bp, Artificial Sequence
  Synthetic oligonucleotide
acattgggactgagacacgg

SEQ ID NO: 91 - DNA, 20 bp, Artificial Sequence
  Synthetic oligonucleotide
aggcttaccaaggcgatgat

SEQ ID NO: 92 - DNA, 20 bp, Artificial Sequence
  Synthetic oligonucleotide
cggcttaccaaggcaatgat

SEQ ID NO: 93 - DNA, 25 bp, Artificial Sequence
  Synthetic oligonucleotide
tgcattagctagttggtaaggtaac

SEQ ID NO: 94 - DNA, 20 bp, Artificial Sequence
  Synthetic oligonucleotide
acattgggactgagacacgg

SEQ ID NO: 95 - DNA, 20 bp, Artificial Sequence
  Synthetic oligonucleotide
aggcttaccaaggcgatgat

SEQ ID NO: 96 - DNA, 20 bp, Artificial Sequence
  Synthetic oligonucleotide
cggcttaccaaggcaatgat

SEQ ID NO: 97 - DNA, 22 bp, Artificial Sequence
  Synthetic oligonucleotide
cgagcttgcctagatgaatttg

SEQ ID NO: 98 - DNA, 27 bp, Artificial Sequence
  Synthetic oligonucleotide
gcctatagaaattcttcggaatggaca

SEQ ID NO: 99 - DNA, 26 bp, Artificial Sequence
  Synthetic oligonucleotide
gatttacttcggtaatgacgttagga

SEQ ID NO: 100 - DNA, 20 bp, Artificial Sequence
  Synthetic oligonucleotide
ctctagacatgcgtctagtg

SEQ ID NO: 101 - DNA, 24 bp, Artificial Sequence
  Synthetic oligonucleotide
caaatggtatcccagacttaaggg

SEQ ID NO: 102 - DNA, 23 bp, Artificial Sequence
  Synthetic oligonucleotide
agctgatcatgcgatctgctttc

SEQ ID NO: 103 - DNA, 19 bp, Artificial Sequence
  Synthetic oligonucleotide
cggcggatgggtgagtaac

SEQ ID NO: 104 - DNA, 19 bp, Artificial Sequence
  Synthetic oligonucleotide
cggcggatgggtgagtaac

SEQ ID NO: 105 - DNA, 23 bp, Artificial Sequence
  Synthetic oligonucleotide
ccaagagactgggataacacctg

SEQ ID NO: 106 - DNA, 20 bp, Artificial Sequence
  Synthetic oligonucleotide
cgcatctgctaaggatgttg

SEQ ID NO: 107 - DNA, 20 bp, Artificial Sequence
  Synthetic oligonucleotide
cagcaatcttttcgccaact

SEQ ID NO: 108 - DNA, 24 bp, Artificial Sequence
  Synthetic oligonucleotide
tgcaactatttctgcagcagatcc

SEQ ID NO: 109 - DNA, 21 bp, Artificial Sequence
  Synthetic oligonucleotide
caggcttggcatattgtccat

SEQ ID NO: 110 - DNA, 24 bp, Artificial Sequence
  Synthetic oligonucleotide
cccaggtgctcttttccgtgctga

SEQ ID NO: 111 - DNA, 24 bp, Artificial Sequence
  Synthetic oligonucleotide
cccaggtgcgctgttccgcgctga

SEQ ID NO: 112 - DNA, 18 bp, Artificial Sequence
  Synthetic oligonucleotide
ggcggcgaaagtgctgtc

SEQ ID NO: 113 - DNA, 25 bp, Artificial Sequence
  Synthetic oligonucleotide
ttcagcgcccaaccaagagctctgt

SEQ ID NO: 114 - DNA, 25 bp, Artificial Sequence
  Synthetic oligonucleotide
ttaagcatccaactaagagctctgt

SEQ ID NO: 115 - DNA, 28 bp, Artificial Sequence
  Synthetic oligonucleotide
tcttcggaatggacatagatacaagcta

SEQ ID NO: 116 - DNA, 16 bp, Artificial Sequence
  Synthetic oligonucleotide
atccgccgctcgcttt

SEQ ID NO: 117 - DNA, 17 bp, Artificial Sequence
  Synthetic oligonucleotide
cgggtgggaaattcggt

SEQ ID NO: 118 - DNA, 18 bp, Artificial Sequence
  Synthetic oligonucleotide
caatgatcggtatcgggt

SEQ ID NO: 119 - DNA, 25 bp, Artificial Sequence
  Synthetic oligonucleotide
cagcttgtagtaaagaattactcac

SEQ ID NO: 120 - DNA, 21 bp, Artificial Sequence
  Synthetic oligonucleotide
ttcgcatattgcactaaatag

SEQ ID NO: 121 - DNA, 21 bp, Artificial Sequence
  Synthetic oligonucleotide
ttcgcatattgcactaaacag

SEQ ID NO: 122 - DNA, 19 bp, Artificial Sequence
  Synthetic oligonucleotide
caacgccaacgaagacaag

SEQ ID NO: 123 - DNA, 19 bp, Artificial Sequence
  Synthetic oligonucleotide
ccagctttgtttgcatcaa

SEQ ID NO: 124 - DNA, 25 bp, Artificial Sequence
  Synthetic oligonucleotide
aaagccgatggtagtagaaaactgc

SEQ ID NO: 125 - DNA, 24 bp, Artificial Sequence
  Synthetic oligonucleotide
ttgaacatctccagtttcaaaggt

SEQ ID NO: 126 - DNA, 22 bp, Artificial Sequence
  Synthetic oligonucleotide
gttggcgttggcaatagctctg

SEQ ID NO: 127 - DNA, 20 bp, Artificial Sequence
  Synthetic oligonucleotide
cgcctcttgatggtgatgat

SEQ ID NO: 128 - DNA, 18 bp, Artificial Sequence
  Synthetic oligonucleotide
tccggtatcacctggctc

SEQ ID NO: 129 - DNA, 30 bp, Artificial Sequence
  Synthetic oligonucleotide
cgttcgtactagagttgtgttgttttggat

SEQ ID NO: 130 - DNA, 27 bp, Artificial Sequence
  Synthetic oligonucleotide
gaggctgtgatgtgtgctgttgaccag

SEQ ID NO: 131 - DNA, 29 bp, Artificial Sequence
  Synthetic oligonucleotide
aggcttgctctttgtcgggcgagcgaacg

SEQ ID NO: 132 - DNA, 23 bp, Artificial Sequence
  Synthetic oligonucleotide
caggtcacagagatttcatcaag

SEQ ID NO: 133 - DNA, 20 bp, Artificial Sequence
  Synthetic oligonucleotide
gaaattcggtggtacgctcc

SEQ ID NO: 134 - DNA, 20 bp, Artificial Sequence
  Synthetic oligonucleotide
gaaattcggtggtactctcc

SEQ ID NO: 135 - DNA, 23 bp, Artificial Sequence
  Synthetic oligonucleotide
gttgtgactctttcaatgcccaa

SEQ ID NO: 136 - DNA, 23 bp, Artificial Sequence
  Synthetic oligonucleotide
gttgtgactctttcaacgctcaa

SEQ ID NO: 137 - DNA, 23 bp, Artificial Sequence
  Synthetic oligonucleotide
gatgtgactccttcaatgctcaa

SEQ ID NO: 138 - DNA, 23 bp, Artificial Sequence
  Synthetic oligonucleotide
gtaagccaacaaagcgtgttctc

SEQ ID NO: 139 - DNA, 23 bp, Artificial Sequence
  Synthetic oligonucleotide
gaaagccaatagagcgtgttctc

SEQ ID NO: 140 - DNA, 19 bp, Artificial Sequence
  Synthetic oligonucleotide
gatcggtatcgggtgcttg

SEQ ID NO: 141 - DNA, 19 bp, Artificial Sequence
  Synthetic oligonucleotide
gatcggtatcgggttcttg

SEQ ID NO: 142 - DNA, 19 bp, Artificial Sequence
  Synthetic oligonucleotide
cagcgtcaccggatttgac

SEQ ID NO: 143 - DNA, 16 bp, Artificial Sequence
  Synthetic oligonucleotide
tgattattgctggtgg

SEQ ID NO: 144 - DNA, 22 bp, Artificial Sequence
  Synthetic oligonucleotide
tgcttgtaaattcgacactttg

SEQ ID NO: 145 - DNA, 23 bp, Artificial Sequence
  Synthetic oligonucleotide
tgtaaattcgacaccttggttga

SEQ ID NO: 146 - DNA, 23 bp, Artificial Sequence
  Synthetic oligonucleotide
ttgtaaattcgacactttggttg

SEQ ID NO: 147 - DNA, 25 bp, Artificial Sequence
  Synthetic oligonucleotide
cgacactttgattgaaaagattgac

SEQ ID NO: 148 - DNA, 21 bp, Artificial Sequence
  Synthetic oligonucleotide
gggtttgcttgaaagacggta

SEQ ID NO: 149 - DNA, 21 bp, Artificial Sequence
  Synthetic oligonucleotide
cgtggtaacttattttaagcg

SEQ ID NO: 150 - DNA, 21 bp, Artificial Sequence
  Synthetic oligonucleotide
gggtttggtgttgagcgatac

SEQ ID NO: 151 - DNA, 25 bp, Artificial Sequence
  Synthetic oligonucleotide
ttgaagatatacgtggtggacgtta

SEQ ID NO: 152 - DNA, 24 bp, Artificial Sequence
  Synthetic oligonucleotide
gcttaagttcagcgggtagtccta

SEQ ID NO: 153 - DNA, 24 bp, Artificial Sequence
  Synthetic oligonucleotide
ggagtttgtaccaatgagtggaaa

SEQ ID NO: 154 - DNA, 27 bp, Artificial Sequence
  Synthetic oligonucleotide
acctaagccattgtcaaagcgatcccg

SEQ ID NO: 155 - DNA, 29 bp, Artificial Sequence
  Synthetic oligonucleotide
tggccaccatttatttcataactttgacc

SEQ ID NO: 156 - DNA, 27 bp, Artificial Sequence
  Synthetic oligonucleotide
ctccgcctttctttcaagcaaacccag

SEQ ID NO: 157 - DNA, 16 bp, Artificial Sequence
  Synthetic oligonucleotide
ggcaacggctgggaat

SEQ ID NO: 158 - DNA, 16 bp, Artificial Sequence
  Synthetic oligonucleotide
agcaacggctgggaat

SEQ ID NO: 159 - DNA, 18 bp, Artificial Sequence
  Synthetic oligonucleotide
caatgatcggtatcgggt

SEQ ID NO: 160 - DNA, 25 bp, Artificial Sequence
  Synthetic oligonucleotide
taaagcctcaccacgattttgacac

SEQ ID NO: 161 - DNA, 22 bp, Artificial Sequence
  Synthetic oligonucleotide
cccaaaaatggccgtaagtatg

SEQ ID NO: 162 - DNA, 24 bp, Artificial Sequence
  Synthetic oligonucleotide
ctgcttgaaagaaatatcggagac

SEQ ID NO: 163 - DNA, 31 bp, Artificial Sequence
  Synthetic oligonucleotide
cgactggttgacgataatcagaggagatggg

SEQ ID NO: 164 - DNA, 17 bp, Artificial Sequence
  Synthetic oligonucleotide
acccaccaaaggctgct

SEQ ID NO: 165 - DNA, 19 bp, Artificial Sequence
  Synthetic oligonucleotide
cgacccaccaaaggctgct

SEQ ID NO: 166 - DNA, 20 bp, Artificial Sequence
  Synthetic oligonucleotide
actgtcacaccgcccacatt

SEQ ID NO: 167 - DNA, 18 bp, Artificial Sequence
  Synthetic oligonucleotide
atagagtagctcggtccc

SEQ ID NO: 168 - DNA, 19 bp, Artificial Sequence
  Synthetic oligonucleotide
tagtgatcggtatcgagtt

SEQ ID NO: 169 - DNA, 18 bp, Artificial Sequence
  Synthetic oligonucleotide
cggtatcgagtttccatg

SEQ ID NO: 170 - DNA, 24 bp, Artificial Sequence
  Synthetic oligonucleotide
ccaaagttgtacaagcaagtacca

SEQ ID NO: 171 - DNA, 22 bp, Artificial Sequence
  Synthetic oligonucleotide
gagccacggtaaagaatacaca

SEQ ID NO: 172 - DNA, 20 bp, Artificial Sequence
  Synthetic oligonucleotide
tttaaagtgacccggatacc

SEQ ID NO: 173 - DNA, 21 bp, Artificial Sequence
  Synthetic oligonucleotide
ctttggatggtcttcaacaga

SEQ ID NO: 174 - DNA, 17 bp, Artificial Sequence
  Synthetic oligonucleotide
atcaccagacttgacgg

SEQ ID NO: 175 - DNA, 20 bp, Artificial Sequence
  Synthetic oligonucleotide
agtctgttgaagaccatcca

SEQ ID NO: 176 - DNA, 22 bp, Artificial Sequence
  Synthetic oligonucleotide
atgtaagttcgacgaattaatc

SEQ ID NO: 177 - DNA, 20 bp, Artificial Sequence
  Synthetic oligonucleotide
tctggcaagatcaaggacat

SEQ ID NO: 178 - DNA, 19 bp, Artificial Sequence
  Synthetic oligonucleotide
gaagattctggcaagatca

SEQ ID NO: 179 - DNA, 21 bp, Artificial Sequence
  Synthetic oligonucleotide
catctgtaacgacaatgcagc

SEQ ID NO: 180 - DNA, 15 bp, Artificial Sequence
  Synthetic oligonucleotide
gacaatgcagcggat

SEQ ID NO: 181 - DNA, 20 bp, Artificial Sequence
  Synthetic oligonucleotide
aactacccacgccaggacat

SEQ ID NO: 182 - DNA, 18 bp, Artificial Sequence
  Synthetic oligonucleotide
ccgcaactacccacgcca